European Patent Specification EP 3 758 735 B1, published December 13, 2023. Title: BIFUNCTIONAL PROTEINS COMBINING CHECKPOINT BLOCKADE FOR TARGETED THERAPY. Applicant: HER, JENG-HORNG. The sequence listing filed with the application follows.

SEQUENCE LISTING (27 sequences)

SEQ ID NO: 1 - protein, 732 aa, Homo sapiens
SKLKDPELSLKGTQHIMQAGQTLHLQCRGEAAHKWSLPEMVSKESERLSITKSACGRNGKQFCSTLTLNTAQANHTGFYSCKYLAVPTSKKKETESAIYIFISDTGRPFVEMYSEIPEIIHMTEGRELVIPCRVTSPNITVTLKKFPLDTLIPDGKRIIWDSRKGFIISNATYKEIGLLTCEATVNGHLYKTNYLTHRQTNTIIDVQISTPRPVKLLRGHTLVLNCTATTPLNTRVQMTWSYPDEKNKRASVRRRIDQSNSHANIFYSVLTIDKMQNKDKGLYTCRVRSGPSFKSVNTSVHIYDKAFITVKHRKQQVLETVAGKRSYRLSMKVKAFPSPEVVWLKDGLPATEKSARYLTRGYSLIIKDVTEEDAGNYTILLSIKQSNVFKNLTATLIVNVKPQIYEKAVSSFPDPALYPLGSRQILTCTAYGIPQPTIKWFWHPCNHNHSEARCDFCSNNEESFILDADSNMGNRIESITQRMAIIEGKNKMASTLVVADSRISGIYICIASNKVGTVGRNISFYITDVPNGFHVNLEKMPTEGEDLKLSCTVNKFLYRDVTWILLRTVNNRTMHYSISKQKMAITKEHSITLNLTIMNVSLQDSGTYACRARNVYTGEEILQKKEITIRDQEAPYLLRNLSDHTVAISSSTTLDCHANGVPEPQITWFKNNHKIQQEPGIILGPGSSTLFIERVTEEDEGVYHCKATNQKGSVESSAYLTVQGTSDKSNLE

SEQ ID NO: 2 - protein, 745 aa, Homo sapiens
ASVGLPSVSLDLPRLSIQKDILTIKANTTLQITCRGQRDLDWLWPNNQSGSEQRVEVTECSDGLFCKTLTIPKVIGNDTGAYKCFYRETDLASVIYVYVQDYRSPFIASVSDQHGVVYITENKNKTVVIPCLGSISNLNVSLCARYPEKRFVPDGNRISWDSKKGFTIPSYMISYAGMVFCEAKINDESYQSIMYIVVVVGYRIYDVVLSPSHGIELSVGEKLVLNCTARTELNVGIDFNWEYPSSKHQHKKLVNRDLKTQSGSEMKKFLSTLTIDGVTRSDQGLYTCAASSGLMTKKNSTFVRVHEKPFVAFGSGMESLVEATVGERVRIPAKYLGYPPPEIKWYKNGIPLESNHTIKAGHVLTIMEVSERDTGNYTVILTNPISKEKQSHVVSLVVYVPPQIGEKSLISPVDSYQYGTTQTLTCTVYAIPPPHHIHWYWQLEEECANEPSQAVSVTNPYPCEEWRSVEDFQGGNKIEVNKNQFALIEGKNKTVSTLVIQAANVSALYKCEAVNKVGRGERVISFHVTRGPEITLQPDMQPTEQESVSLWCTADRSTFENLTWYKLGPQPLPIHVGELPTPVCKNLDTLWKLNATMFSNSTNDILIMELKNASLQDQGDYVCLAQDRKTKKRHCVVRQLTVLERVAPTITGNLENQTTSIGESIEVSCTASGNPPPQIMWFKDNETLVEDSGIVLKDGNRNLTIRRVRKEDEGLYTCQACSVLGCAKVEAFFIIEGAQEKTNLE

SEQ ID NO: 3 - protein, 217 aa, Homo sapiens
QSVLTQPPSASGTPGQRVTISCSGSSSNIGSNTVNWYQQLPGTAPKLLIYSNNQRPSGVPDRFSGSKSGTSASLAISGLQSEDEADYYCATWDDSLNAWVVFGGGTKLTVLGQPKAAPSVTLFPPSSEELQANKATLVCLISDFYPGAVTVAWKADSSPVKAGVETTTPSKQSNNKYAASSYLSLTPEQWKSHRSYSCQVTHEGSTVEKTVAPTECS

SEQ ID NO: 4 - protein, 118 aa, Homo sapiens
QVQLVQSGAEVKKPGSSVKVSCKASGGTFRRYSISWVRQAPGQGLEWMGGIIPVFGAAKYAQKFQGRVTITADEFTSTAYMELSSLTSEDTAVYYCALSGDSDAFDIWGQGTMVTVSS

SEQ ID NO: 5 - protein, 216 aa, Homo sapiens
QSALTQPASVSGSPGQSITISCTGTSNDVGSYNSVSWYQQHPGKAPKLVIYEVANRPSGVPDRFSGSKSGNTASLTISGLQAEDEADYYCSSYTSSSTLVFGGGTKLTVLGQPKAAPSVTLFPPSSEELQANKATLVCLISDFYPGAVTVAWKADSSPVKAGVETTTPSKQSNNKYAASSYLSLTPEQWKSHRSYSCQVTHEGSTVEKTVAPTECS

SEQ ID NO: 6 - protein, 121 aa, Homo sapiens
QVQLVQSGAKVKKPGSSVKVSCKASGGTFSSYAISWVRQAPGQGLEWMGRIIPILGIANYAQKFQGRVTITADKSTSTAYMELSSLRSEDTAVYYCARVVPGYSYGPFDYWGQGTTVTVSS

SEQ ID NO: 7 - protein, 328 aa, Homo sapiens
ASTKGPSVFPLAPCSRSTSESTAALGCLVKDYFPEPVTVSWNSGALTSGVHTFPAVLQSSGLYSLSSVVTVPSSSLGTKTYTCNVDHKPSNTKVDKRVESKYGPPCPPCPAPEFLGGPSVFLFPPKPKDTLMISRTPEVTCVVVDVSQEDPEVQFNWYVDGVEVHNAKTKPREEQFNSTYRVVSVLTVLHQDWLNGKEYKCKVSNKGLPSSIEKTISKAKGQPREPQVYTLPPSQEEMTKNQVSLTCLVKGFYPSDIAVEWESNGQPENNYKTTPPVLDSDGSFFLYSRLTVDKSRWQEGNVFSCSVMHEALHNHYTQKSLSLSLGGG

SEQ ID NO: 8 - protein, 329 aa, Artificial Sequence
  constant domain in heavy chain of engineered IgG1 (eIgG1)
ASTKGPSVFPLAPSSKSTSGGTAALGCLVKDYFPEPVTVSWNSGALTSGVHTFPAVLQSSGLYSLSSVVTVPSSSLGTQTYICNVNHKPSNTKVDKKVEPKSCDKTHTCPPCPAPELLGGPSVFLFPPKPKDTLMISRTPEVTCVVVDVSHEDPEVKFNWYVDGVEVHNAKTKPREEQYASTYRVVSVLTVLHQDWLNGKEYKCAVSNKALPAPIEKTISKAKGQPREPQVYTLPPSREEMTKNQVSLTCLVKGFYPSDIAVEWESNGQPENNYKTTPPVLDSDGSFFLYSKLTVDKSRWQQGNVFSCSVMHEALHNHYTQKSLSLSPG

SEQ ID NO: 9 - protein, 205 aa, Homo sapiens
GDTGRPFVEMYSEIPEIIHMTEGRELVIPCRVTSPNITVTLKKFPLDTLIPDGKRIIWDSRKGFIISNATYKEIGLLTCEATVNGHLYKTNYLTHRQTNTIIDVVLSPSHGIELSVGEKLVLNCTARTELNVGIDFNWEYPSSKHQHKKLVNRDLKTQSGSEMKKFLSTLTIDGVTRSDQGLYTCAASSGLMTKKNSTFVRVHEK

SEQ ID NO: 10 - protein, 5 aa, Artificial Sequence
  peptide linker
GGGGS

SEQ ID NO: 11 - protein, 20 aa, Artificial Sequence
  signal peptide
METDTLLLWVLLLWVPGSTG

SEQ ID NO: 12 - protein, 666 aa, Artificial Sequence
  Anti-PD-L1-clone 6 Heavy Chain -VID/IgG4 bispecific antibody
QVQLVQSGAEVKKPGSSVKVSCKASGGTFRRYSISWVRQAPGQGLEWMGGIIPVFGAAKYAQKFQGRVTITADEFTSTAYMELSSLTSEDTAVYYCALSGDSDAFDIWGQGTMVTVSSASTKGPSVFPLAPCSRSTSESTAALGCLVKDYFPEPVTVSWNSGALTSGVHTFPAVLQSSGLYSLSSVVTVPSSSLGTKTYTCNVDHKPSNTKVDKRVESKYGPPCPPCPAPEFLGGPSVFLFPPKPKDTLMISRTPEVTCVVVDVSQEDPEVQFNWYVDGVEVHNAKTKPREEQFNSTYRVVSVLTVLHQDWLNGKEYKCKVSNKGLPSSIEKTISKAKGQPREPQVYTLPPSQEEMTKNQVSLTCLVKGFYPSDIAVEWESNGQPENNYKTTPPVLDSDGSFFLYSRLTVDKSRWQEGNVFSCSVMHEALHNHYTQKSLSLSLGGGGGGGSGGGGSGGGGSGDTGRPFVEMYSEIPEIIHMTEGRELVIPCRVTSPNITVTLKKFPLDTLIPDGKRIIWDSRKGFIISNATYKEIGLLTCEATVNGHLYKTNYLTHRQTNTIIDVVLSPSHGIELSVGEKLVLNCTARTELNVGIDFNWEYPSSKHQHKKLVNRDLKTQSGSEMKKFLSTLTIDGVTRSDQGLYTCAASSGLMTKKNSTFVRVHEK

SEQ ID NO: 13 - protein, 669 aa, Artificial Sequence
  Anti-PD-L1-clone 6 Heavy Chain -VID/eIgG1 bispecific antibody
QVQLVQSGAEVKKPGSSVKVSCKASGGTFRRYSISWVRQAPGQGLEWMGGIIPVFGAAKYAQKFQGRVTITADEFTSTAYMELSSLTSEDTAVYYCALSGDSDAFDIWGQGTMVTVSSASTKGPSVFPLAPSSKSTSGGTAALGCLVKDYFPEPVTVSWNSGALTSGVHTFPAVLQSSGLYSLSSVVTVPSSSLGTQTYICNVNHKPSNTKVDKKVEPKSCDKTHTCPPCPAPELLGGPSVFLFPPKPKDTLMISRTPEVTCVVVDVSHEDPEVKFNWYVDGVEVHNAKTKPREEQYASTYRVVSVLTVLHQDWLNGKEYKCAVSNKALPAPIEKTISKAKGQPREPQVYTLPPSREEMTKNQVSLTCLVKGFYPSDIAVEWESNGQPENNYKTTPPVLDSDGSFFLYSKLTVDKSRWQQGNVFSCSVMHEALHNHYTQKSLSLSPGGGGGGGSGGGGSGGGGSGDTGRPFVEMYSEIPEIIHMTEGRELVIPCRVTSPNITVTLKKFPLDTLIPDGKRIIWDSRKGFIISNATYKEIGLLTCEATVNGHLYKTNYLTHRQTNTIIDVVLSPSHGIELSVGEKLVLNCTARTELNVGIDFNWEYPSSKHQHKKLVNRDLKTQSGSEMKKFLSTLTIDGVTRSDQGLYTCAASSGLMTKKNSTFVRVHEK

SEQ ID NO: 14 - protein, 49 aa, Homo sapiens
PELSLKGTQHIMQAGQTLHLQCRGEAAHKWSLPEMVSKESERLSITKSA

SEQ ID NO: 15 - protein, 64 aa, Homo sapiens
GRELVIPCRVTSPNITVTLKKFPLDTLIPDGKRIIWDSRKGFIISNATYKEIGLLTCEATVNGH

SEQ ID NO: 16 - protein, 98 aa, Homo sapiens
IDVQISTPRPVKLLRGHTLVLNCTATTPLNTRVQMTWSYPDEKNKRASVRRRIDQSNSHANIFYSVLTIDKMQNKDKGLYTCRVRSGPSFKSVNTSVH

SEQ ID NO: 17 - protein, 87 aa, Homo sapiens
TVKHRKQQVLETVAGKRSYRLSMKVKAFPSPEVVWLKDGLPATEKSARYLTRGYSLIIKDVTEEDAGNYTILLSIKQSNVFKNLTAT

SEQ ID NO: 18 - protein, 126 aa, Homo sapiens
PQIYEKAVSSFPDPALYPLGSRQILTCTAYGIPQPTIKWFWHPCNHNHSEARCDFCSNNEESFILDADSNMGNRIESITQRMAIIEGKNKMASTLVVADSRISGIYICIASNKVGTVGRNISFYIT

SEQ ID NO: 19 - protein, 94 aa, Homo sapiens
PNGFHVNLEKMPTEGEDLKLSCTVNKFLYRDVTWILLRTVNNRTMHYSISKQKMAITKEHSITLNLTIMNVSLQDSGTYACRARNVYTGEEILQ

SEQ ID NO: 20 - protein, 87 aa, Homo sapiens
PYLLRNLSDHTVAISSSTTLDCHANGVPEPQITWFKNNHKIQQEPGIILGPGSSTLFIERVTEEDEGVYHCKATNQKGSVESSAYLT

SEQ ID NO: 21 - protein, 65 aa, Homo sapiens
NTTLQITCRGQRDLDWLWPNNQSGSEQRVEVTECSDGLFCKTLTIPKVIGNDTGAYKCFYRETDL

SEQ ID NO: 22 - protein, 67 aa, Homo sapiens
NKNKTVVIPCLGSISNLNVSLCARYPEKRFVPDGNRISWDSKKGFTIPSYMISYAGMVFCEAKINDE

SEQ ID NO: 23 - protein, 97 aa, Homo sapiens
YDVVLSPSHGIELSVGEKLVLNCTARTELNVGIDFNWEYPSSKHQHKKLVNRDLKTQSGSEMKKFLSTLTIDGVTRSDQGLYTCAASSGLMTKKNST

SEQ ID NO: 24 - protein, 86 aa, Homo sapiens
FVAFGSGMESLVEATVGERVRIPAKYLGYPPPEIKWYKNGIPLESNHTIKAGHVLTIMEVSERDTGNYTVILTNPISKEKQSHVVS

SEQ ID NO: 25 - protein, 128 aa, Homo sapiens
PQIGEKSLISPVDSYQYGTTQTLTCTVYAIPPPHHIHWYWQLEEECANEPSQAVSVTNPYPCEEWRSVEDFQGGNKIEVNKNQFALIEGKNKTVSTLVIQAANVSALYKCEAVNKVGRGERVISFHVT

SEQ ID NO: 26 - protein, 110 aa, Homo sapiens
PEITLQPDMQPTEQESVSLWCTADRSTFENLTWYKLGPQPLPIHVGELPTPVCKNLDTLWKLNATMFSNSTNDILIMELKNASLQDQGDYVCLAQDRKTKKRHCVVRQLT

SEQ ID NO: 27 - protein, 87 aa, Homo sapiens
PTITGNLENQTTSIGESIEVSCTASGNPPPQIMWFKDNETLVEDSGIVLKDGNRNLTIRRVRKEDEGLYTCQACSVLGCAKVEAFFI